European Patent Specification EP 3 272 770 B1, published December 20, 2023. Title: BINDING MOLECULES. Applicant: CRAIG, Roger Kingdon. The sequence listing filed with the application follows.

SEQUENCE LISTING (35 sequences)

SEQ ID NO: 1 - DNA, 39 bp, Artificial Sequence
  PCR primer
aatctgggcagcggccgcctcgacacaacatttgcgctc

SEQ ID NO: 2 - DNA, 318 bp, Human HCAb (IgG3) against rtTA
agactctcctgtgcagcctctggaagcatcttcagtatcaatgccatgggctggtaccgccaggctccagggaagcagcgcgagttggtcgcagctattactagtggtggtagcacaaggtatgcagactccgtgaagggccgattcaccatctccagagacaacgccaagaacacggtgtatctgcaaatgaacagcctgaaacctgaggacacggccgtctattactgtttgatctctatggttcggggagcccgttttgactactggggccagggaaccctggtcaccgtctcctcagagctcaaaaccccactt

SEQ ID NO: 3 - protein, 106 aa, Human HCAb (IgG3) against rtTA
RLSCAASGSIFSINAMGWYRQAPGKQRELVAAITSGGSTRYADSVKGRFTISRDNAKNTVYLQMNSLKPEDTAVYYCLISMVRGARFDYWGQGTLVTVSSELKTPL

SEQ ID NO: 4 - DNA, 33 bp, Artificial Sequence
  PCR primer
ctggaattctcaaccatggagctggggctgagc

SEQ ID NO: 5 - DNA, 30 bp, Artificial Sequence
  PCR primer
gacaagctttacccggagacagggagaggc

SEQ ID NO: 6 - DNA, 30 bp, Artificial Sequence; identical to SEQ ID NO: 5
  PCR primer

SEQ ID NO: 7 - DNA, 34 bp, Artificial Sequence
  PCR primer
gtcctcgaggcccaggtccaactgcaggagtctg

SEQ ID NO: 8 - DNA, 37 bp, Artificial Sequence
  PCR primer
gtcgaattctcattccgaggagacggtgacctgggtc

SEQ ID NO: 9 - DNA, 36 bp, IgG Hinge sequence
gagcgcaaatgttgtgtcgagtgcccaccgtgccca

SEQ ID NO: 10 - DNA, 44 bp, Replacement IgG hinge sequence
agcttctgagcgcaaaccaccagtcgagccaccaccgccaccac

SEQ ID NO: 11 - DNA, 44 bp, Complement of replacement IgG hinge sequence
tcgagtggtggcggtggtggctcgactggtggtttgcgctcaga

SEQ ID NO: 12 - DNA, 404 bp, VDJg*1
gacacggccgtgtagtatctgtaaggcagatggggtagtactatggttcggggagtccaccactgcggctagaggggccagggaacactggtcgcggtgtcatcagcctccaccaagggcccatcggtcttccccctggcgccctgctccaggagcacctccgagagcacagcggccctgggctgcctggtcaaggactacttccccgaaccggtgacggtgtcgtggaactcaggcgctctgaccagcggcgtgcacaccttcccagctgtcctacagtcctcaggactctactccctcagcagcgtggtgaccgtgccctccagcaacttcggcacccagacctacacctgcaacgtagatcacaagcccagcaacaccaagagcgcaaatgttgtgtcgag

SEQ ID NO: 13 - DNA, 352 bp, VDJg*2
gacattcccacttcgatctctggggccgtggcaccctggtcactgtctcctcagcctccaccaagggcccatcggtcttccccctggcgccctgctccaggagcacctccgagagcacagcggccctgggctgcctggtcaaggactacttccccgaaccggtgacggtgtcgtggaactcaggcgctctgaccagcggcgtgcacaccttcccagctgtcctacagtcctcaggactctactccctcagcagcgtggtgaccgtgccctccagcaacttcggcacccagacctacacctgcaacgtagatcacaagcccagcaacaccaagagcgcaaatgttgtgtcgag

SEQ ID NO: 14 - DNA, 394 bp, VDJg*3
gacacggccgtctattactgtaatgccactacgatattttgactggttattatagacgctactggggccagggaaccctggtcaccgtctcctcagcctccgccaagggcccatcggtcttccccctggcgccctgctccaggagcacctccgagagcacagcggccctgggctgcctggtcaaggactacttccccgaaccggtgacggtgtcgtggaactcaggcgctctgaccagcggcgtgcacaccttcccagctgtcctacagtcctcaggactctactccctcagcagcgtggtgaccgtgccctccagcaacttcggcacccagacctacacctgcaacgtagatcacaagcccagcaacaccaagagcgcaaatgttgtgtcgag

SEQ ID NO: 15 - DNA, 380 bp, VDJg*4
gacacggccgtccaatcggatacagctatggttacgtactttgactactggggccagggaaccctggtcaccgtctcctcagcctccaccaagggcccatcggtcttccccctggcgccctgctccaggagcacctccgagagcacagcggccctgggctgcctggtcaaggactacttccccgaaccggtgacggtgtcgtggaactcaggcgctctgaccagcggcgtgcacaccttcccagctgtcctacagtcctcaggactctactccctcagcagcgtggtgaccgtgccctccagcaacttcggcacccagacctacacctgcaacgtagatcacaagcccagcaacaccaagagcgcaaatgttgtgtcgag

SEQ ID NO: 16 - DNA, 417 bp, VDJg*5
gacacggccgtctattactgtaatgcagatgtattactatggttcggggagcctatagccttactactactacggtatggacgtctggggccaagggaccacggtcaccgtctcctcagcctccaccaagggcccatcggtcttccccctggcgccctgctccaggagcacctccgagagcacagcggccctgggctgcctggtcaaggactacttccccgaaccggtgacggtgtcgtggaactcaggcgctctgaccagcggcgtgcacaccttcccagctgtcctacagtcctcaggactctactccctcagcagcgtggtgaccgtgccctccagcaacttcggcacccagacctacacctgcaacgtagatcacaagcccagcaacaccaagagcgcaaatgttgtgtcgag

SEQ ID NO: 17 - protein, 108 aa, alpha-B.pertussis 1
RLSCAASGSIFSINAMGWYRQAPGKQRELVAAITSGGSTNYADSVKGRFTISRDNAKNTVYLQMNSLKPEDTAVYYCNAKGPITHVRGVHYWGQGTLVTVSSERKCCV

SEQ ID NO: 18 - protein, 108 aa, alpha-B.pertussis 2
RLSCAASGSIFSINAMGWYRQAPGKQRELVAAITSGGSTNYADSVKGRFTISRDNAKNTVYLQMNSLKPEDTAVYYCNAKTPITHIRGVHHWGQGTLVTVSSERKCCV

SEQ ID NO: 19 - protein, 108 aa, alpha-B.pertussis 3
RLSCAASGSIFSINAMGWYRQAPGKQRELVAAITSGGSTNYADSVKGRFTISRDNAKNTVYLQMNSLKPEDTAVYYCNARTPITVVRGVHYWGQGTLVTVSSERKCCV

SEQ ID NO: 20 - protein, 108 aa, alpha-B.pertussis 4
RLSCAASGSIFSINAMGWYRQAPGKQRELVAAITSGGSTNYADSVKGRFTISRDKAKNTVYLQMNSLKPEDSAVYYCNRTGPITHVRGVDYWGRGTLVTVSSERKCCV

SEQ ID NO: 21 - protein, 108 aa, alpha-B.pertussis 5
RLSCAASGSIFSINAMGWYRQAPGKQRELVAAITSGGSTNHADSVKGRFTISRDNAKNTVYLQMNSLKPEDTAVYYCNAESPITKVRGVSYWGQGTLVTVSSERKCCV

SEQ ID NO: 22 - protein, 59 aa, neVHH1 original
RLSCAASGFTLDYYAIGWFRQAEGKEREGVSCISSSDGSTYYADSVKGRFTISRDNAKN

SEQ ID NO: 23 - protein, 59 aa, neVHH1 clone 1; identical to SEQ ID NO: 22

SEQ ID NO: 24 - protein, 59 aa, neVHH1 clone 2
RLSCAASGFTLDYYVIGWFRQAEGKEREGVSCISSSDGSTYYADSVKGRFTISRDNAKN

SEQ ID NO: 25 - protein, 59 aa, neVHH1 clone 3
RLSCAASGFTLDYYAIGWFRQAEGKEREGVSCISSSDGSTYYGDSVKGRFTISRDKAKN

SEQ ID NO: 26 - protein, 58 aa, neVHH2 original
RLSCAASGSIFSINAMGWYRQAPGKQRELVAAITSGGSTNYADSVKGRFTISRDNAKN

SEQ ID NO: 27 - protein, 58 aa, neVHH2 clone 1
RLSCAASGSIFSINAMGWYRQAPGKQRELVAAITSGGSTKYADSVKGRFTISRDNAKN

SEQ ID NO: 28 - protein, 58 aa, neVHH2 clone 2
RLSCAASGSIFSINVMGWYRQPPGKQRELVAGVTSGGSTSYADSVKGRFTISRDNAKN

SEQ ID NO: 29 - protein, 58 aa, neVHH2 clone 3
RLSCAASGSIFSINAMGWYRQAPGKQRELVAPITSGGSTNYADSVKGRFTISRDNAKN

SEQ ID NO: 30 - protein, 78 aa, VHH2 germline
RLSCAASGSIFSINAMGWYRQAPGKQRELVAAITSGGSTNYADSVKGRFTISRDNAKNTVYLQMNSLKPEDTAVYYCN

SEQ ID NO: 31 - protein, 105 aa, alpha-Tetanus 1
RLSCAASGSIFSINAMGWYRQAPGKQRELVAAITSGGSTNYADSVKGRFTISRDNAKNTVYLQMNSLKPEDTAVYYCNAERAGDPFDYWGQGTLVTVSSERKCCV

SEQ ID NO: 32 - protein, 108 aa, alpha-Tetanus 2
RLSCAASGSIFSINAMGWYRQAPGKQRELVAAITSGGSTNYADSVKGRFTISRDNAKNTVYLQMNSLKPEDTAVYYCGVLWFGELSDWFDYWGQGTLVTVSSERKCCV

SEQ ID NO: 33 - protein, 108 aa, alpha-Tetanus 3
RLSCAASGSIFSINAMGWYRQAPGKQRELVAAITSGGSTNYADSVKGRFTISRDNAKNTVYLQMNSLKPEDTAVYYCNADCWGSRWYFDHYWGRGTLVTVSSERKCCV

SEQ ID NO: 34 - protein, 111 aa, alpha-Tetanus 4
RLSCAASGSIFSINAMGWYRQAPGKQRELVAAITSGGSTNYADSVKGRFTISRDNAKNTVYLQMNSLKPEDTAVYYCNADTSPPRYFDWLPFDYWGQGTLVTVSSERKCCV

SEQ ID NO: 35 - protein, 112 aa, alpha-hsp70
RLSCAASGSIFSSNAMGWSRQAPGKQRELVAAITSGGSTNYADSVKGRFTISRDNAKNTVHLQMNSLKPEDTAVYYCNAGNTMVRGVIIKYRFDYWGQGTLVTVSSERKCCV